European Patent Specification EP 3 711 741 B1, published April 30, 2025. Title: METHOD FOR MANUFACTURING BONE GRAFT COMPOSITE AND BONE GRAFT COMPOSITE MANUFACTURED THEREBY. Applicant: KOREA TOOTH BANK CO.,LTD. Application KRPCT/KR2018/002067. The sequence listing filed with the application follows.

SEQUENCE LISTING (2 sequences)

SEQ ID NO: 1 - DNA, 34 bp, primer sequence
  sense primer
agaagaacatatgcaagccaaacacaaacagcgg

SEQ ID NO: 2 - DNA, 33 bp, primer sequence
  antisense primer
aattttacagcttctagcgacacccacaaccct